European Patent Specification EP 3 644 722 B1, published December 11, 2024. Title: NON-HUMAN ANIMALS COMPRISING A HUMANIZED ASGR1 LOCUS. Applicant: Regeneron Pharmaceuticals, Inc. Mujica, Alejo Gusarova, Viktoria Wang, Cheng Kyratsous, Christos Potocky, Terra Cygnar, Katherine Martin, Joel. The sequence listing filed with the application follows.

SEQUENCE LISTING (42 sequences)

SEQ ID NO: 1 - protein, 291 aa, Homo sapiens
  MISC_FEATURE (1)..(40): Cytoplasmic Domain
  MISC_FEATURE (41)..(61): Transmembrane Domain
  MISC_FEATURE (61)..(123): Coiled-Coil Domain
  MISC_FEATURE (161)..(278): C-Type Lectin Domain
MTKEYQDLQHLDNEESDHHQLRKGPPPPQPLLQRLCSGPRLLLLSLGLSLLLLVVVCVIGSQNSQLQEELRGLRETFSNFTASTEAQVKGLSTQGGNVGRKMKSLESQLEKQQKDLSEDHSSLLLHVKQFVSDLRSLSCQMAALQGNGSERTCCPVNWVEHERSCYWFSRSGKAWADADNYCRLEDAHLVVVTSWEEQKFVQHHIGPVNTWMGLHDQNGPWKWVDGTDYETGFKNWRPEQPDDWYGHGLGGGEDCAHFTDDGRWNDDVCQRPYRWVCETELDKASQEPPLL

SEQ ID NO: 2 - protein, 284 aa, Mus musculus
  MISC_FEATURE (1)..(39): Cytoplasmic Domain
  MISC_FEATURE (40)..(60): Transmembrane Domain
  MISC_FEATURE (60)..(122): Coiled-Coil Domain
  MISC_FEATURE (160)..(277): C-Type Lectin Domain
MTKDYQDFQHLDNDNDHHQLRRGPPPTPRLLQRLCSGSRLLLLSSSLSILLLVVVCVITSQNSQLREDLLALRQNFSNLTVSTEDQVKALSTQGSSVGRKMKLVESKLEKQQKDLTEDHSSLLLHVKQLVSDVRSLSCQMAAFRGNGSERTCCPINWVEYEGSCYWFSSSVRPWTEADKYCQLENAHLVVVTSRDEQNFLQRHMGPLNTWIGLTDQNGPWKWVDGTDYETGFQNWRPEQPDNWYGHGLGGGEDCAHFTTDGRWNDDVCRRPYRWVCETKLDKAN

SEQ ID NO: 3 - protein, 290 aa, Artificial Sequence
  Synthetic
  MISC_FEATURE (1)..(39): Cytoplasmic Domain
  MISC_FEATURE (40)..(60): Transmembrane Domain
  MISC_FEATURE (60)..(122): Coiled-Coil Domain
  MISC_FEATURE (62)..(290): Residues Encoded by Introduced Human Exons
  MISC_FEATURE (160)..(277): C-Type Lectin Domain
MTKDYQDFQHLDNDNDHHQLRRGPPPTPRLLQRLCSGSRLLLLSSSLSILLLVVVCVITSQNSQLQEELRGLRETFSNFTASTEAQVKGLSTQGGNVGRKMKSLESQLEKQQKDLSEDHSSLLLHVKQFVSDLRSLSCQMAALQGNGSERTCCPVNWVEHERSCYWFSRSGKAWADADNYCRLEDAHLVVVTSWEEQKFVQHHIGPVNTWMGLHDQNGPWKWVDGTDYETGFKNWRPEQPDDWYGHGLGGGEDCAHFTDDGRWNDDVCQRPYRWVCETELDKASQEPPLL

SEQ ID NO: 4 - DNA, 855 bp, Mus musculus
atgacaaaggattatcaagatttccagcacctggacaatgataatgaccatcatcaactccggagagggccgcctcccactccacggctcttgcagcgactctgctctggatcccgcctcctcctgctctcctcgagcctcagcattctgttgctggtggttgtctgtgtgatcacatcccaaaattcccaactccgggaagatctgctggctctaaggcagaatttcagcaacctcactgtgagcactgaggaccaggtcaaggccctgagcacccagggaagtagtgtgggaagaaagatgaagttagtggagtcgaagctggaaaaacagcagaaggatctgactgaagatcactccagtttgctactgcacgtgaagcagttagtgtctgacgtgcgaagcttgagctgccagatggctgcatttcggggcaatggctctgaaaggacctgctgccccatcaactgggtggagtatgaaggcagctgctactggttctccagctctgtgaggccttggactgaagctgacaagtactgccagctggaaaatgcccatctggtggtggtgacctccagggatgagcagaacttcctccagcgccacatgggccccttaaacacttggattggcctaactgaccagaacgggccctggaaatgggtggatggaacagactacgagacaggcttccagaattggagaccagagcagccagataactggtacggacatgggcttggaggaggcgaggactgtgcccacttcacgacggatggccgctggaatgacgacgtctgcaggaggccctaccgctgggtctgtgagacaaagttggataaggctaattag

SEQ ID NO: 5 - DNA, 876 bp, Homo sapiens
atgaccaaggagtatcaagaccttcagcatctggacaatgaggagagtgaccaccatcagctcagaaaagggccacctcctccccagcccctcctgcagcgtctctgctccggacctcgcctcctcctgctctccctgggcctcagcctcctgctgcttgtggttgtctgtgtgatcggatcccaaaactcccagctgcaggaggagctgcggggcctgagagagacgttcagcaacttcacagcgagcacggaggcccaggtcaagggcttgagcacccagggaggcaatgtgggaagaaagatgaagtcgctagagtcccagctggagaaacagcagaaggacctgagtgaagatcactccagcctgctgctccacgtgaagcagttcgtgtctgacctgcggagcctgagctgtcagatggcggcgctccagggcaatggctcagaaaggacctgctgcccggtcaactgggtggagcacgagcgcagctgctactggttctctcgctccgggaaggcctgggctgacgccgacaactactgccggctggaggacgcgcacctggtggtggtcacgtcctgggaggagcagaaatttgtccagcaccacataggccctgtgaacacctggatgggcctccacgaccaaaacgggccctggaagtgggtggacgggacggactacgagacgggcttcaagaactggaggccggagcagccggacgactggtacggccacgggctcggaggaggcgaggactgtgcccacttcaccgacgacggccgctggaacgacgacgtctgccagaggccctaccgctgggtctgcgagacagagctggacaaggccagccaggagccacctctcctttaa

SEQ ID NO: 6 - DNA, 19 bp, Artificial Sequence
  Synthetic
tcccaactccgggaagatc

SEQ ID NO: 7 - DNA, 24 bp, Artificial Sequence
  Synthetic
tgctggctctaaggcagaatttca

SEQ ID NO: 8 - DNA, 20 bp, Artificial Sequence
  Synthetic
tcagtgctcacagtgaggtt

SEQ ID NO: 9 - DNA, 22 bp, Artificial Sequence
  Synthetic
gggttggctcatgttaggaagg

SEQ ID NO: 10 - DNA, 20 bp, Artificial Sequence
  Synthetic
tcagcagccgagctgtgaaa

SEQ ID NO: 11 - DNA, 22 bp, Artificial Sequence
  Synthetic
caggctgtgctacccaaagttc

SEQ ID NO: 12 - DNA, 21 bp, Artificial Sequence
  Synthetic
ggaggcaatgtgggaagaaag

SEQ ID NO: 13 - DNA, 24 bp, Artificial Sequence
  Synthetic
tgaagtcgctagagtcccagctgg

SEQ ID NO: 14 - DNA, 20 bp, Artificial Sequence
  Synthetic
tcaggtccttctgctgtttc

SEQ ID NO: 15 - DNA, 20 bp, Artificial Sequence
  Synthetic
gattgggaatccgcccatct

SEQ ID NO: 16 - DNA, 29 bp, Artificial Sequence
  Synthetic
cctcttctgctttctcgggaattttcatc

SEQ ID NO: 17 - DNA, 20 bp, Artificial Sequence
  Synthetic
aaagcgccacgggtttcaag

SEQ ID NO: 18 - DNA, 120 bp, Artificial Sequence
  Synthetic
  misc_feature (1)..(60): Mouse Sequence
  misc_feature (61)..(120): Human Sequence
catcccaaagtgggtggccagggctgggcagagaaagggggcaacttcgggtgtgtgtgacaagggagtggtgggtgcagtggtggcggacacagcgatcccgttttcttctctctgcac

SEQ ID NO: 19 - DNA, 160 bp, Artificial Sequence
  Synthetic
  misc_feature (1)..(60): Human Sequence
  misc_feature (61)..(66): XhoI
  misc_feature (67)..(100): loxP
  misc_feature (101)..(160): Cassette
tgttatttacagatacgtgagtttgggcaaattattgttctctgtgtcccagctgtaaacctcgagataacttcgtataatgtatgctatacgaagttatatgcatggcctccgcgccgggttttggcgcctcccgcgggcgcccccctcctcacggcga

SEQ ID NO: 20 - DNA, 191 bp, Artificial Sequence
  Synthetic
  misc_feature (1)..(60): Cassette
  misc_feature (61)..(94): loxP
  misc_feature (100)..(125): I-CeuI
  misc_feature (126)..(131): NheI
  misc_feature (132)..(191): Mouse Sequence
tttcactgcattctagttgtggtttgtccaaactcatcaatgtatcttatcatgtctggaataacttcgtataatgtatgctatacgaagttatgctagtaactataacggtcctaaggtagcgagctagccgtggacagatacagcaacgtgagctagttattctgtcctaaagtctcagttggaagatg

SEQ ID NO: 21 - DNA, 9692 bp, Artificial Sequence
  Synthetic
  misc_feature (1)..(69): Mouse Sequence
  misc_feature (70)..(3976): Human Sequence
  misc_feature (3977)..(3982): XhoI
  misc_feature (3983)..(4016): loxP
  misc_feature (4023)..(5235): Human Ubiquitin Promoter
  misc_feature (5236)..(5302): EM7 Promoter
  misc_feature (5303)..(6328): Hygromycin Resistance Gene
  misc_feature (6329)..(6813): PGK polyA
  misc_feature (6825)..(7506): Prm Promoter
  misc_feature (7507)..(8646): Crei
  misc_feature (8909)..(9119): SV40 polyA
  misc_feature (9124)..(9157): loxP
  misc_feature (9163)..(9188): I-CeuI
  misc_feature (9189)..(9194): NheI
  misc_feature (9195)..(9692): Mouse Sequence
gtgtgatcacatcccaaagtgggtggccagggctgggcagagaaagggggcaacttcgggtgtgtgtgacaagggagtggtgggtgcagtggtggcggacacagcgatcccgttttcttctctctgcacgctgtcctggccagactcccagctgcaggaggagctgcggggcctgagagagacgttcagcaacttcacagcgagcacggaggcccaggtcaagggcttgagcacccagggtgagggcgctggggcggggctggggctggggctggggctggggggctgtcgggaacgctgagcgagcctctcccgcaggaggcaatgtgggaagaaagatgaagtcgctagagtcccagctggagaaacagcagaaggacctgagtgaaggtcagagagggagtgtgtgtgtgtgtgtgtgtgtgtgaaagagagtgagaatgtgtggatgtgtgtgagaaagtgtgagtgtgtgtggatgtgtgtgagaatgagagggagtgtgtgtgtgtgtgagtctgtgtgtgagaatgagggggagtgtgttttgggtgtgtgtatgagagccttgtgtggatgtgagaatgagagggagtgtgtatgtctgtgagtgtgagaatgagatggagtgtgtgtgagtctgtgtgtgagaatgaggtgtgtgtgtgtgagaatgagatggtgtgtgtgtgggaatgagagggggtgtgtgtctgagtgtgagaatgagatagagtgtgtgtgagacagtctgtgggaatgagagggagtgtgtgtgagagtgtgagaatgacggagtgtgtctgtgagtgtgataatgaggtgtgtgtgagtctgagtgtaagaatgagatggggtgtgtgtgtctgtgagtgtgagagtgtgagaatgaggggtgtttgtgtctgagtgtgagtctgtgagtgtgagaatgagatggggtgtgtgagtgagtgtgagaatgagatggggtgtgtgtgtctgtgagtgtgtgtgtgtttgtgagtgtgagaatgagatggggtgtgtgtgagtgtgagaatgagatggggtgtgtgtctgtgtgtgagaatgagatgggtgtgtgtgtgacagagtctgagtgtgagaatgagagggagtgtgtgtgagtgtgagaatgagaaggagtggatgggtgtgtgagtctgtgtgaatgagggagtgggtgtgtgtacgagtgtgagtctgtgtttatgtgtgagaatgtgtcagtgtatgtgtgtgagaacgtgtgtatgtgtgttagtgtgtgttgcgtgtgtgggggaatgagagggattgtgtctgtgagtgtgagaatgagatggagtgtctgtgagactgtgtgtgaggagtgggagtgtgtgtgagaatgagatgggtgtgtgtgtctgagtgtgtgtctgtgagaatgagagggagtgtgtgtgtgtgtgagagcctgtgtgaaaatgagaaggagtgtggatgggtgtttgtgagtgggagagtctgtgtgtttatgtgtgtgagaatgagggagtgtgggtgtgtgtgcgaatgtgagtctgtgtttatgtgtgtgagaatgtgtcagtgtatgtgagaacgtgtgtgttagtgtgttgcgtgtgtgagaatgtaagtatatgtgtaagtgcatgtgagtgtgtgtatgtgcgtgttgtgtgaatgtgcattgtgtgtgcatgtgtgaaagagtatatgtgtgttgtgggtgagtgtgtgtggtgtgtgtagtgggtgagggtgtgttgtatgtgtgggtgtgcgttgtgtgaatgtgtgtatgtgggtgagggtgtgtgtgcctgtgtgagggtgtgttgtggtttttgtgtgtgtttgggtgagggtgtgttgtgtgtgtgtgtgggtgaaggtgtgttgtgtgtgtcgtgggtgaaggtgtgttgtgtgtgtagtgactgtagattagggtgtgttccgtgtgtgtgtgtgagggtgtatgttgtgggtgttttgtgtgtgagtgggtgtgtaagggtgtgttgtgtgtatgtgggttaaggtgtgttatgcgtgagggtgtattgtgtgtgtgttttgtgtgtgttgtgtgtatgtgggttagggtgtgttgtgtgtttgtgtgttttgtgtgttgtctgtgtatgtgggttacggtgtgttgtgcgtgtgagggtgtgttgtgtatggtgtgttgtgtgtgttgtgtgagtgtgtatgtgagttagggtgtgttgtgtctatgtatgtgtgtgtaagggtgtgttgtgtgtctgtgggtgtgttttgtgtatgtgggttagggtgtgttgtgtgttctgtattgtgtgttttatgtgttgtctgtatgtgggttatgtgtgttgtgtgtgttgtggatgtatgtgggttagggtgtgttgtgtgtctctgtgtgttgtctgcgtttgtgtctgtgggttagggtgtgttgtatgtgttgtgttttgtgtgttgtccgtgtgtgtgtatgtgggttaggttgtgtgtgtgtgtgttgtatattgtctgtgtgtgtgtgttaggatgtgttgtgtgtctgtgtgagtgtgtgtgtaagggtgtgttgtgtgtgtaggagtgtgtgtgtgtgtgtgtatgggggtctctcaggccaactccgctgctgtttgtggcaatgcgacgggtgttcgggtcccagcaggaggatgtagggctgacctcgtttcccgtttccctccccgtggtttccgcatctcctcccgctcccctccgcccggtctccccagatcactccagcctgctgctccacgtgaagcagttcgtgtctgacctgcggagcctgagctgtcagatggcggcgctccagggcaatggtaaggaggccagcccggcccgctctctgcctccccccttctctgggcagcgcttagcccctgcgccccgtttctcccgctcaggctcagaaaggacctgctgcccggtcaactgggtggagcacgagcgcagctgctactggttctctcgctccgggaaggcctgggctgacgccgacaactactgccggctggaggacgcgcacctggtggtggtcacgtcctgggaggagcaggtgaggacccggagggtctgggaggctggctggcctcggagagatcaccacccgccttctctctcctcagaaatttgtccagcaccacataggccctgtgaacacctggatgggcctccacgaccaaaacgggccctggaagtgggtggacgggacggactacgagacgggcttcaagtgagtgcgcgccctccctcggcctgggtccggccgccttcgcgccctggggccctgggctgaggagtctggagcgacccgcctgcggatccgacctcctggggcccacagctggctctgtccccaggaactggaggccggagcagccggacgactggtacggccacgggctcggaggaggcgaggactgtgcccacttcaccgacgacggccgctggaacgacgacgtctgccagaggccctaccgctgggtctgcgagacagagctggacaaggccagccaggagccacctctcctttaatttatttcttcaatgcctcgacctgccgcaggggtccgggattgggaatccgcccatctgggggcctcttctgctttctcgggaattttcatctaggattttaagggaaggggaaggatagggtgatgttccgaaggtgaggagcttgaaacccgtggcgctttctgcagtttgcaggttatcattgtgaactttttttttttaagagtaaaaagaaatatacctaaaccttctgttagttgtctggttattggggattcggaagcaggagtgggctggttggcattacgaagccttagcgggtgctgtggcatcatgagaactgtgtgggctttgggccagaatggccagactttgttatttacagatacgtgagtttgggcaaattattgttctctgtgtcccagctgtaaacctcgagataacttcgtataatgtatgctatacgaagttatatgcatggcctccgcgccgggttttggcgcctcccgcgggcgcccccctcctcacggcgagcgctgccacgtcagacgaagggcgcagcgagcgtcctgatccttccgcccggacgctcaggacagcggcccgctgctcataagactcggccttagaaccccagtatcagcagaaggacattttaggacgggacttgggtgactctagggcactggttttctttccagagagcggaacaggcgaggaaaagtagtcccttctcggcgattctgcggagggatctccgtggggcggtgaacgccgatgattatataaggacgcgccgggtgtggcacagctagttccgtcgcagccgggatttgggtcgcggttcttgtttgtggatcgctgtgatcgtcacttggtgagtagcgggctgctgggctggccggggctttcgtggccgccgggccgctcggtgggacggaagcgtgtggagagaccgccaagggctgtagtctgggtccgcgagcaaggttgccctgaactgggggttggggggagcgcagcaaaatggcggctgttcccgagtcttgaatggaagacgcttgtgaggcgggctgtgaggtcgttgaaacaaggtggggggcatggtgggcggcaagaacccaaggtcttgaggccttcgctaatgcgggaaagctcttattcgggtgagatgggctggggcaccatctggggaccctgacgtgaagtttgtcactgactggagaactcggtttgtcgtctgttgcgggggcggcagttatggcggtgccgttgggcagtgcacccgtacctttgggagcgcgcgccctcgtcgtgtcgtgacgtcacccgttctgttggcttataatgcagggtggggccacctgccggtaggtgtgcggtaggcttttctccgtcgcaggacgcagggttcgggcctagggtaggctctcctgaatcgacaggcgccggacctctggtgaggggagggataagtgaggcgtcagtttctttggtcggttttatgtacctatcttcttaagtagctgaagctccggttttgaactatgcgctcggggttggcgagtgtgttttgtgaagttttttaggcaccttttgaaatgtaatcatttgggtcaatatgtaattttcagtgttagactagtaaattgtccgctaaattctggccgtttttggcttttttgttagacgtgttgacaattaatcatcggcatagtatatcggcatagtataatacgacaaggtgaggaactaaaccatgaaaaagcctgaactcaccgcgacgtctgtcgagaagtttctgatcgaaaagttcgacagcgtgtccgacctgatgcagctctcggagggcgaagaatctcgtgctttcagcttcgatgtaggagggcgtggatatgtcctgcgggtaaatagctgcgccgatggtttctacaaagatcgttatgtttatcggcactttgcatcggccgcgctcccgattccggaagtgcttgacattggggaattcagcgagagcctgacctattgcatctcccgccgtgcacagggtgtcacgttgcaagacctgcctgaaaccgaactgcccgctgttctgcagccggtcgcggaggccatggatgcgattgctgcggccgatcttagccagacgagcgggttcggcccattcggaccgcaaggaatcggtcaatacactacatggcgtgatttcatatgcgcgattgctgatccccatgtgtatcactggcaaactgtgatggacgacaccgtcagtgcgtccgtcgcgcaggctctcgatgagctgatgctttgggccgaggactgccccgaagtccggcacctcgtgcacgcggatttcggctccaacaatgtcctgacggacaatggccgcataacagcggtcattgactggagcgaggcgatgttcggggattcccaatacgaggtcgccaacatcttcttctggaggccgtggttggcttgtatggagcagcagacgcgctacttcgagcggaggcatccggagcttgcaggatcgccgcggctccgggcgtatatgctccgcattggtcttgaccaactctatcagagcttggttgacggcaatttcgatgatgcagcttgggcgcagggtcgatgcgacgcaatcgtccgatccggagccgggactgtcgggcgtacacaaatcgcccgcagaagcgcggccgtctggaccgatggctgtgtagaagtactcgccgatagtggaaaccgacgccccagcactcgtccgagggcaaaggaatagggggatccgctgtaagtctgcagaaattgatgatctattaaacaataaagatgtccactaaaatggaagtttttcctgtcatactttgttaagaagggtgagaacagagtacctacattttgaatggaaggattggagctacgggggtgggggtggggtgggattagataaatgcctgctctttactgaaggctctttactattgctttatgataatgtttcatagttggatatcataatttaaacaagcaaaaccaaattaagggccagctcattcctcccactcatgatctatagatctatagatctctcgtgggatcattgtttttctcttgattcccactttgtggttctaagtactgtggtttccaaatgtgtcagtttcatagcctgaagaacgagatcagcagcctctgttccacatacacttcattctcagtattgttttgccaagttctaattccatcagacctcgacctgcagcccctagcccgggcgccagtagcagcacccacgtccaccttctgtctagtaatgtccaacacctccctcagtccaaacactgctctgcatccatgtggctcccatttatacctgaagcacttgatggggcctcaatgttttactagagcccacccccctgcaactctgagaccctctggatttgtctgtcagtgcctcactggggcgttggataatttcttaaaaggtcaagttccctcagcagcattctctgagcagtctgaagatgtgtgcttttcacagttcaaatccatgtggctgtttcacccacctgcctggccttgggttatctatcaggacctagcctagaagcaggtgtgtggcacttaacacctaagctgagtgactaactgaacactcaagtggatgccatctttgtcacttcttgactgtgacacaagcaactcctgatgccaaagccctgcccacccctctcatgcccatatttggacatggtacaggtcctcactggccatggtctgtgaggtcctggtcctctttgacttcataattcctaggggccactagtatctataagaggaagagggtgctggctcccaggccacagcccacaaaattccacctgctcacaggttggctggctcgacccaggtggtgtcccctgctctgagccagctcccggccaagccagcaccatgggtacccccaagaagaagaggaaggtgcgtaccgatttaaattccaatttactgaccgtacaccaaaatttgcctgcattaccggtcgatgcaacgagtgatgaggttcgcaagaacctgatggacatgttcagggatcgccaggcgttttctgagcatacctggaaaatgcttctgtccgtttgccggtcgtgggcggcatggtgcaagttgaataaccggaaatggtttcccgcagaacctgaagatgttcgcgattatcttctatatcttcaggcgcgcggtctggcagtaaaaactatccagcaacatttgggccagctaaacatgcttcatcgtcggtccgggctgccacgaccaagtgacagcaatgctgtttcactggttatgcggcggatccgaaaagaaaacgttgatgccggtgaacgtgcaaaacaggctctagcgttcgaacgcactgatttcgaccaggttcgttcactcatggaaaatagtgatcgctgccaggatatacgtaatctggcatttctggggattgcttataacaccctgttacgtatagccgaaattgccaggatcagggttaaagatatctcacgtactgacggtgggagaatgttaatccatattggcagaacgaaaacgctggttagcaccgcaggtgtagagaaggcacttagcctgggggtaactaaactggtcgagcgatggatttccgtctctggtgtagctgatgatccgaataactacctgttttgccgggtcagaaaaaatggtgttgccgcgccatctgccaccagccagctatcaactcgcgccctggaagggatttttgaagcaactcatcgattgatttacggcgctaaggtaaatataaaatttttaagtgtataatgtgttaaactactgattctaattgtttgtgtattttaggatgactctggtcagagatacctggcctggtctggacacagtgcccgtgtcggagccgcgcgagatatggcccgcgctggagtttcaataccggagatcatgcaagctggtggctggaccaatgtaaatattgtcatgaactatatccgtaacctggatagtgaaacaggggcaatggtgcgcctgctggaagatggcgattgatctagataagtaatgatcataatcagccatatcacatctgtagaggttttacttgctttaaaaaacctcccacacctccccctgaacctgaaacataaaatgaatgcaattgttgttgttaaacctgccctagttgcggccaattccagctgagcgtgcctccgcaccattaccagttggtctggtgtcaaaaataataataaccgggcaggggggatctaagctctagataagtaatgatcataatcagccatatcacatctgtagaggttttacttgctttaaaaaacctcccacacctccccctgaacctgaaacataaaatgaatgcaattgttgttgttaacttgtttattgcagcttataatggttacaaataaagcaatagcatcacaaatttcacaaataaagcatttttttcactgcattctagttgtggtttgtccaaactcatcaatgtatcttatcatgtctggaataacttcgtataatgtatgctatacgaagttatgctagtaactataacggtcctaaggtagcgagctagccgtggacagatacagcaacgtgagctagttattctgtcctaaagtctcagttggaagatgggaggatttttgacctctgtctgctgggggcaggaccaaccaccagggaactgcagcccccctgtgctgagtgcatcagagacttggaatggaacacactggcctgcgacactcatcacaacgaacagaaactgctttgtacactgaataaacgcagtgaatacccagctcaggatcacagacacatgaatgcaaagttatattagtataaccaagggtgggaatgagggcaattacagataacttatagacatgaattactaacaaaacagggcaaaatgtttgctcataaataacatgaaaatacaatatatagtcatatgtatatatacatgtatatatataaatgacataatatgtatatatttttacaaatacactgcaggaaaataatatttttcctctacagaagagattggcaaatctgacatctaaaat

SEQ ID NO: 22 - DNA, 160 bp, Artificial Sequence
  Synthetic
  misc_feature (1)..(90): Mouse Sequence
  misc_feature (91)..(160): Human Sequence
catgatgtttctttcttaggaaagccagggcatttctctattctccaatctcttggctcaatgcccttggcctctcttttgttccactagtgaagcctctccagccaggggctgaggtcccggtggtgtgggcccaggagggggctcctgcccagctccc

SEQ ID NO: 23 - DNA, 197 bp, Artificial Sequence
  Synthetic
  misc_feature (1)..(60): Human Sequence
  misc_feature (61)..(66): XhoI
  misc_feature (67)..(100): loxP
  misc_feature (106)..(131): I-CeuI
  misc_feature (132)..(137): NheI
  misc_feature (138)..(197): Mouse Sequence
tgttatttacagatacgtgagtttgggcaaattattgttctctgtgtcccagctgtaaacctcgagataacttcgtataatgtatgctatacgaagttatgctagtaactataacggtcctaaggtagcgagctagccgtggacagatacagcaacgtgagctagttattctgtcctaaagtctcagttggaagatg

SEQ ID NO: 24 - DNA, 4551 bp, Artificial Sequence
  Synthetic
  misc_feature (1)..(69): Mouse Sequence
  misc_feature (70)..(3976): Human Sequence
  misc_feature (3977)..(3982): XhoI
  misc_feature (3983)..(4016): LoxP
  misc_feature (4022)..(4047): I-CeuI
  misc_feature (4048)..(4053): NheI
  misc_feature (4054)..(4551): Mouse Sequence
gtgtgatcacatcccaaagtgggtggccagggctgggcagagaaagggggcaacttcgggtgtgtgtgacaagggagtggtgggtgcagtggtggcggacacagcgatcccgttttcttctctctgcacgctgtcctggccagactcccagctgcaggaggagctgcggggcctgagagagacgttcagcaacttcacagcgagcacggaggcccaggtcaagggcttgagcacccagggtgagggcgctggggcggggctggggctggggctggggctggggggctgtcgggaacgctgagcgagcctctcccgcaggaggcaatgtgggaagaaagatgaagtcgctagagtcccagctggagaaacagcagaaggacctgagtgaaggtcagagagggagtgtgtgtgtgtgtgtgtgtgtgtgaaagagagtgagaatgtgtggatgtgtgtgagaaagtgtgagtgtgtgtggatgtgtgtgagaatgagagggagtgtgtgtgtgtgtgagtctgtgtgtgagaatgagggggagtgtgttttgggtgtgtgtatgagagccttgtgtggatgtgagaatgagagggagtgtgtatgtctgtgagtgtgagaatgagatggagtgtgtgtgagtctgtgtgtgagaatgaggtgtgtgtgtgtgagaatgagatggtgtgtgtgtgggaatgagagggggtgtgtgtctgagtgtgagaatgagatagagtgtgtgtgagacagtctgtgggaatgagagggagtgtgtgtgagagtgtgagaatgacggagtgtgtctgtgagtgtgataatgaggtgtgtgtgagtctgagtgtaagaatgagatggggtgtgtgtgtctgtgagtgtgagagtgtgagaatgaggggtgtttgtgtctgagtgtgagtctgtgagtgtgagaatgagatggggtgtgtgagtgagtgtgagaatgagatggggtgtgtgtgtctgtgagtgtgtgtgtgtttgtgagtgtgagaatgagatggggtgtgtgtgagtgtgagaatgagatggggtgtgtgtctgtgtgtgagaatgagatgggtgtgtgtgtgacagagtctgagtgtgagaatgagagggagtgtgtgtgagtgtgagaatgagaaggagtggatgggtgtgtgagtctgtgtgaatgagggagtgggtgtgtgtacgagtgtgagtctgtgtttatgtgtgagaatgtgtcagtgtatgtgtgtgagaacgtgtgtatgtgtgttagtgtgtgttgcgtgtgtgggggaatgagagggattgtgtctgtgagtgtgagaatgagatggagtgtctgtgagactgtgtgtgaggagtgggagtgtgtgtgagaatgagatgggtgtgtgtgtctgagtgtgtgtctgtgagaatgagagggagtgtgtgtgtgtgtgagagcctgtgtgaaaatgagaaggagtgtggatgggtgtttgtgagtgggagagtctgtgtgtttatgtgtgtgagaatgagggagtgtgggtgtgtgtgcgaatgtgagtctgtgtttatgtgtgtgagaatgtgtcagtgtatgtgagaacgtgtgtgttagtgtgttgcgtgtgtgagaatgtaagtatatgtgtaagtgcatgtgagtgtgtgtatgtgcgtgttgtgtgaatgtgcattgtgtgtgcatgtgtgaaagagtatatgtgtgttgtgggtgagtgtgtgtggtgtgtgtagtgggtgagggtgtgttgtatgtgtgggtgtgcgttgtgtgaatgtgtgtatgtgggtgagggtgtgtgtgcctgtgtgagggtgtgttgtggtttttgtgtgtgtttgggtgagggtgtgttgtgtgtgtgtgtgggtgaaggtgtgttgtgtgtgtcgtgggtgaaggtgtgttgtgtgtgtagtgactgtagattagggtgtgttccgtgtgtgtgtgtgagggtgtatgttgtgggtgttttgtgtgtgagtgggtgtgtaagggtgtgttgtgtgtatgtgggttaaggtgtgttatgcgtgagggtgtattgtgtgtgtgttttgtgtgtgttgtgtgtatgtgggttagggtgtgttgtgtgtttgtgtgttttgtgtgttgtctgtgtatgtgggttacggtgtgttgtgcgtgtgagggtgtgttgtgtatggtgtgttgtgtgtgttgtgtgagtgtgtatgtgagttagggtgtgttgtgtctatgtatgtgtgtgtaagggtgtgttgtgtgtctgtgggtgtgttttgtgtatgtgggttagggtgtgttgtgtgttctgtattgtgtgttttatgtgttgtctgtatgtgggttatgtgtgttgtgtgtgttgtggatgtatgtgggttagggtgtgttgtgtgtctctgtgtgttgtctgcgtttgtgtctgtgggttagggtgtgttgtatgtgttgtgttttgtgtgttgtccgtgtgtgtgtatgtgggttaggttgtgtgtgtgtgtgttgtatattgtctgtgtgtgtgtgttaggatgtgttgtgtgtctgtgtgagtgtgtgtgtaagggtgtgttgtgtgtgtaggagtgtgtgtgtgtgtgtgtatgggggtctctcaggccaactccgctgctgtttgtggcaatgcgacgggtgttcgggtcccagcaggaggatgtagggctgacctcgtttcccgtttccctccccgtggtttccgcatctcctcccgctcccctccgcccggtctccccagatcactccagcctgctgctccacgtgaagcagttcgtgtctgacctgcggagcctgagctgtcagatggcggcgctccagggcaatggtaaggaggccagcccggcccgctctctgcctccccccttctctgggcagcgcttagcccctgcgccccgtttctcccgctcaggctcagaaaggacctgctgcccggtcaactgggtggagcacgagcgcagctgctactggttctctcgctccgggaaggcctgggctgacgccgacaactactgccggctggaggacgcgcacctggtggtggtcacgtcctgggaggagcaggtgaggacccggagggtctgggaggctggctggcctcggagagatcaccacccgccttctctctcctcagaaatttgtccagcaccacataggccctgtgaacacctggatgggcctccacgaccaaaacgggccctggaagtgggtggacgggacggactacgagacgggcttcaagtgagtgcgcgccctccctcggcctgggtccggccgccttcgcgccctggggccctgggctgaggagtctggagcgacccgcctgcggatccgacctcctggggcccacagctggctctgtccccaggaactggaggccggagcagccggacgactggtacggccacgggctcggaggaggcgaggactgtgcccacttcaccgacgacggccgctggaacgacgacgtctgccagaggccctaccgctgggtctgcgagacagagctggacaaggccagccaggagccacctctcctttaatttatttcttcaatgcctcgacctgccgcaggggtccgggattgggaatccgcccatctgggggcctcttctgctttctcgggaattttcatctaggattttaagggaaggggaaggatagggtgatgttccgaaggtgaggagcttgaaacccgtggcgctttctgcagtttgcaggttatcattgtgaactttttttttttaagagtaaaaagaaatatacctaaaccttctgttagttgtctggttattggggattcggaagcaggagtgggctggttggcattacgaagccttagcgggtgctgtggcatcatgagaactgtgtgggctttgggccagaatggccagactttgttatttacagatacgtgagtttgggcaaattattgttctctgtgtcccagctgtaaacctcgagataacttcgtataatgtatgctatacgaagttatgctagtaactataacggtcctaaggtagcgagctagccgtggacagatacagcaacgtgagctagttattctgtcctaaagtctcagttggaagatgggaggatttttgacctctgtctgctgggggcaggaccaaccaccagggaactgcagcccccctgtgctgagtgcatcagagacttggaatggaacacactggcctgcgacactcatcacaacgaacagaaactgctttgtacactgaataaacgcagtgaatacccagctcaggatcacagacacatgaatgcaaagttatattagtataaccaagggtgggaatgagggcaattacagataacttatagacatgaattactaacaaaacagggcaaaatgtttgctcataaataacatgaaaatacaatatatagtcatatgtatatatacatgtatatatataaatgacataatatgtatatatttttacaaatacactgcaggaaaataatatttttcctctacagaagagattggcaaatctgacatctaaaat

SEQ ID NO: 25 - protein, 10 aa, Artificial Sequence
  Synthetic
EQKLISEEDL

SEQ ID NO: 26 - DNA, 30 bp, Artificial Sequence
  Synthetic
gaacaaaaactcatctcagaagaggatctg

SEQ ID NO: 27 - protein, 63 aa, Homo sapiens
SQNSQLQEELRGLRETFSNFTASTEAQVKGLSTQGGNVGRKMKSLESQLEKQQKDLSEDHSSL

SEQ ID NO: 28 - protein, 118 aa, Homo sapiens
HERSCYWFSRSGKAWADADNYCRLEDAHLVVVTSWEEQKFVQHHIGPVNTWMGLHDQNGPWKWVDGTDYETGFKNWRPEQPDDWYGHGLGGGEDCAHFTDDGRWNDDVCQRPYRWVCE

SEQ ID NO: 29 - protein, 39 aa, Mus musculus
MTKDYQDFQHLDNDNDHHQLRRGPPPTPRLLQRLCSGSR

SEQ ID NO: 30 - protein, 21 aa, Mus musculus
LLLLSSSLSILLLVVVCVITS

SEQ ID NO: 31 - protein, 229 aa, Homo sapiens
NSQLQEELRGLRETFSNFTASTEAQVKGLSTQGGNVGRKMKSLESQLEKQQKDLSEDHSSLLLHVKQFVSDLRSLSCQMAALQGNGSERTCCPVNWVEHERSCYWFSRSGKAWADADNYCRLEDAHLVVVTSWEEQKFVQHHIGPVNTWMGLHDQNGPWKWVDGTDYETGFKNWRPEQPDDWYGHGLGGGEDCAHFTDDGRWNDDVCQRPYRWVCETELDKASQEPPLL

SEQ ID NO: 32 - DNA, 20 bp, Artificial Sequence
  Synthetic
ggagtaccagctcccgtacg

SEQ ID NO: 33 - DNA, 43 bp, Artificial Sequence
  Synthetic
ctcttctgagatgagtttttgttcgttgcctctctggaggttg

SEQ ID NO: 34 - DNA, 43 bp, Artificial Sequence
  Synthetic
aaactcatctcagaagaggatctgagacaagcagctaccgcag

SEQ ID NO: 35 - DNA, 18 bp, Artificial Sequence
  Synthetic
tccgcccgctgtttaaac

SEQ ID NO: 36 - DNA, 21 bp, Artificial Sequence
  Synthetic
ggaacccctagtgatggagtt

SEQ ID NO: 37 - DNA, 16 bp, Artificial Sequence
  Synthetic
cggcctcagtgagcga

SEQ ID NO: 38 - DNA, 21 bp, Artificial Sequence
  Synthetic
cactccctctctgcgcgctcg

SEQ ID NO: 39 - protein, 291 aa, Macaca fascicularis
MTKEYQDLQHLDNEESDHHQLGKGPPPPQSLLRRLCSGPRLLLLSLGLSLLLLVVVCVIGSQNAQLQRELRGLRETLSNFTASTEAQVKGLSTQGGNVGRKMKSLESQLEKQQKDLSEDHSSLLLHVKQFVSDLRSLSCQMAALQGNGSERACCPVNWVEHERSCYWFSRSGKAWADADNYCRLEDAHLVVVTSWEEQKFVQHHIGPVNTWMGLHDQNGPWKWVDGTDYETGFKNWRPEQPDDWYGHGLGGGEDCAHFTDDGRWNDDVCQRPYRWVCETELDKASQEPPLL

SEQ ID NO: 40 - DNA, 876 bp, Macaca fascicularis
atgaccaaggagtatcaggacctgcagcatctggacaatgaggagagtgaccaccatcagctcggaaaagggccacctcctccgcagtccctcctgcggcgtctctgctccggccctcgcctcctcctgctctccctgggcctcagcctcctgctgctggtggttgtctgtgtgatcggatcccaaaacgcccagctgcagcgggagctgcggggcctgagagagacgctcagcaacttcacagcgagcaccgaggcccaggtcaagggcttgagcacccagggaggcaatgtgggaagaaagatgaagtcgctggagtcccagctggagaaacagcagaaggacttgagtgaagatcactccagcctgctgctccacgtgaagcagttcgtgtctgacctgcggagcctgagctgtcagatggcggcgctccagggcaatggctcggaaagggcctgctgcccagtcaactgggtggagcacgagcgcagctgctactggttctctcgctccgggaaggcctgggccgacgccgacaactactgccggctggaggacgcgcacctggtggtggtcacgtcctgggaggagcagaaatttgtccagcaccacataggtcctgtgaacacctggatgggcctccacgaccaaaacgggccctggaagtgggtggacgggacggactacgagacgggcttcaagaactggagaccggagcagccggacgactggtacggccacgggctcgggggaggggaggactgtgcccacttcaccgacgacggccgctggaacgacgacgtctgccagaggccctaccgctgggtctgcgagacagagctggacaaggccagtcaggagccacctctcctttaa

SEQ ID NO: 41 - protein, 284 aa, Rattus norvegicus
MTKDYQDFQHLDNENDHHQLQRGPPPAPRLLQRLCSGFRLFLLSLGLSILLLVVVCVITSQNSQLREDLRVLRQNFSNFTVSTEDQVKALTTQGERVGRKMKLVESQLEKHQEDLREDHSRLLLHVKQLVSDVRSLSCQMAALRGNGSERICCPINWVEYEGSCYWFSSSVKPWTEADKYCQLENAHLVVVTSWEEQRFVQQHMGPLNTWIGLTDQNGPWKWVDGTDYETGFKNWRPGQPDDWYGHGLGGGEDCAHFTTDGHWNDDVCRRPYRWVCETELGKAN

SEQ ID NO: 42 - DNA, 855 bp, Rattus norvegicus
atgacaaaggattatcaagatttccagcacttggacaatgagaacgaccaccatcaactccagagagggccacctcccgctccaaggctcttgcagcgactctgctctggattccgtctcttcctgctttccctgggcctcagcatcctgctgctggtggttgtctgtgtgatcacatcccaaaattcccaactccgggaagatctgcgggttctaaggcagaatttcagcaactttaccgtgagcactgaggaccaggtcaaggccctgaccacccagggagagagagtgggaagaaagatgaagttagtcgagtcacagctggaaaaacatcaggaggatctgagggaagaccactctagattgctactgcatgtaaagcagttagtgtctgacgtgcgaagcttgagctgccagatggccgcacttcggggcaatggctctgaaaggatctgctgccccatcaactgggtggagtatgaaggcagctgctactggttctccagctctgtgaagccttggacggaagctgacaagtactgccagctggagaacgcccacctggtggtggtgacttcctgggaggagcagagattcgtccagcaacacatgggccccttaaatacttggattggcctaactgaccagaacggaccctggaaatgggtggatgggacagactatgagacaggcttcaagaactggagaccagggcagccagatgactggtacggacatgggcttggagggggtgaagactgtgcccacttcaccaccgatggccactggaatgatgacgtctgcaggaggccctaccgctgggtctgtgagacagagttgggcaaggccaattag